European Patent Application EP 4 268 944 A2, published November 1, 2023. Title: Analyte Sequencing with Nanopores. Applicant: University of Washington. The sequence listing filed with the application follows.

SEQUENCE LISTING (55 sequences)

SEQ ID NO: 1-3 - skipped (3 entries)

SEQ ID NO: 4 - DNA, 84 bp, synthetic construct
  misc_feature 1..84: note = Synthetic
  source 1..84: mol_type = other DNA
gctggctctgttgctctctcgcaacagagccagcaaaaaaaaaaaaaaaaaaaaaaaaaaaaaaaaaaaaaaaaaaaaaaaaaa

SEQ ID NO: 5 - DNA, 100 bp, synthetic construct
  misc_feature 1..100: note = Synthetic
  source 1..100: mol_type = other DNA
gcaacagagccagccccgcaacagagccagcggagcaacagagccagctttgcaacagagccagcaaaaaaaaaaaaaaaaaaaaaaaaaaaaaaaaaaa

SEQ ID NO: 6 - DNA, 100 bp, synthetic construct
  misc_feature 1..100: note = Synthetic
  source 1..100: mol_type = other DNA
gcaacagagccagcggagcaacagagccagccccgcaacagagccagcaaagcaacagagccagctttaaaaaaaaaaaaaaaaaaaaaaaaaaaaaaaa

SEQ ID NO: 7 - DNA, 100 bp, synthetic construct
  misc_feature 1..100: note = Synthetic
  source 1..100: mol_type = other DNA
gcaacagagccagccccgcaacagagccagcaaagcaacagagccagccccgcaacagagccagctttgcaacagagccagcggaaaaaaaaaaaaaaaa

SEQ ID NO: 8 - DNA, 14 bp, synthetic construct
  misc_feature 1..14: note = Synthetic
  source 1..14: mol_type = other DNA
gctggctctgttgc

SEQ ID NO: 9 - DNA, 180 bp, synthetic construct
  misc_feature 1..180: note = Synthetic
  source 1..180: mol_type = other DNA
gctggctctgttgctctctcgcaacagagccagccccgctggctctgttgctctctcgcaacagagccagcggagctggctctgttgctctctcgcaacagagccagctttgctggctctgttgctctctcgcaacagagccagcaaaaaaaaaaaaaaaaaaaaaaaaaaaaaaaaaaa

SEQ ID NO: 10 - DNA, 50 bp, synthetic construct
  misc_feature 1..50: note = Synthetic
  source 1..50: mol_type = other DNA
aaaaaaaaaaaaaaaaaaaaaaaaaaaaaaaaaaaaaaaaaaaaaaaaaa

SEQ ID NO: 11 - DNA, 50 bp, synthetic construct
  misc_feature 1..50: note = Synthetic
  source 1..50: mol_type = other DNA
cccccccccccccccccccccccccccccccccccccccccccccccccc

SEQ ID NO: 12 - DNA, 50 bp, synthetic construct
  misc_feature 1..50: note = Synthetic
  source 1..50: mol_type = other DNA
tttttttttttttttttttttttttttttttttttttttttttttttttt

SEQ ID NO: 13 - DNA, 47 bp, synthetic construct
  misc_feature 1..47: note = Synthetic
  source 1..47: mol_type = other DNA
aaaaaaaaaaaaaaaaaaaaaaaaaaaaaaaaaaaaaaaaaaaaaaa

SEQ ID NO: 14 - DNA, 50 bp, synthetic construct
  misc_feature 1..50: note = Synthetic
  source 1..50: mol_type = other DNA
gggggggggggggggggggggggggggggggggggggggggggggggggg

SEQ ID NO: 15 - DNA, 50 bp, synthetic construct
  misc_feature 1..50: note = Synthetic
  source 1..50: mol_type = other DNA
caaaaaaaaaaaaaaaaaaaaaaaaaaaaaaaaaaaaaaaaaaaaaaaaa

SEQ ID NO: 16 - DNA, 50 bp, synthetic construct
  misc_feature 1..50: note = Synthetic
  source 1..50: mol_type = other DNA
acaaaaaaaaaaaaaaaaaaaaaaaaaaaaaaaaaaaaaaaaaaaaaaaa

SEQ ID NO: 17 - DNA, 50 bp, synthetic construct
  misc_feature 1..50: note = Synthetic
  source 1..50: mol_type = other DNA
aacaaaaaaaaaaaaaaaaaaaaaaaaaaaaaaaaaaaaaaaaaaaaaaa

SEQ ID NO: 18 - DNA, 50 bp, synthetic construct
  misc_feature 1..50: note = Synthetic
  source 1..50: mol_type = other DNA
accaaaaaaaaaaaaaaaaaaaaaaaaaaaaaaaaaaaaaaaaaaaaaaa

SEQ ID NO: 19 - DNA, 50 bp, synthetic construct
  misc_feature 1..50: note = Synthetic
  source 1..50: mol_type = other DNA
cacaaaaaaaaaaaaaaaaaaaaaaaaaaaaaaaaaaaaaaaaaaaaaaa

SEQ ID NO: 20 - DNA, 50 bp, synthetic construct
  misc_feature 1..50: note = Synthetic
  source 1..50: mol_type = other DNA
ccaaaaaaaaaaaaaaaaaaaaaaaaaaaaaaaaaaaaaaaaaaaaaaaa

SEQ ID NO: 21 - DNA, 50 bp, synthetic construct
  misc_feature 1..50: note = Synthetic
  source 1..50: mol_type = other DNA
taaaaaaaaaaaaaaaaaaaaaaaaaaaaaaaaaaaaaaaaaaaaaaaaa

SEQ ID NO: 22 - DNA, 50 bp, synthetic construct
  misc_feature 1..50: note = Synthetic
  source 1..50: mol_type = other DNA
ataaaaaaaaaaaaaaaaaaaaaaaaaaaaaaaaaaaaaaaaaaaaaaaa

SEQ ID NO: 23 - DNA, 50 bp, synthetic construct
  misc_feature 1..50: note = Synthetic
  source 1..50: mol_type = other DNA
aataaaaaaaaaaaaaaaaaaaaaaaaaaaaaaaaaaaaaaaaaaaaaaa

SEQ ID NO: 24 - DNA, 50 bp, synthetic construct
  misc_feature 1..50: note = Synthetic
  source 1..50: mol_type = other DNA
attttttttttttttttttttttttttttttttttttttttttttttttt

SEQ ID NO: 25 - DNA, 50 bp, synthetic construct
  misc_feature 1..50: note = Synthetic
  source 1..50: mol_type = other DNA
tatttttttttttttttttttttttttttttttttttttttttttttttt

SEQ ID NO: 26 - DNA, 50 bp, synthetic construct
  misc_feature 1..50: note = Synthetic
  source 1..50: mol_type = other DNA
ttattttttttttttttttttttttttttttttttttttttttttttttt

SEQ ID NO: 27 - DNA, 50 bp, synthetic construct
  misc_feature 1..50: note = Synthetic
  source 1..50: mol_type = other DNA
gggaaaaaaaaaaaaaaaaaaaaaaaaaaaaaaaaaaaaaaaaaaaaaaa

SEQ ID NO: 28 - DNA, 50 bp, synthetic construct
  misc_feature 1..50: note = Synthetic
  source 1..50: mol_type = other DNA
ccccaaaaaaaaaaaaaaaaaaaaaaaaaaaaaaaaaaaaaaaaaaaaaa

SEQ ID NO: 29 - DNA, 50 bp, synthetic construct
  misc_feature 1..50: note = Synthetic
  source 1..50: mol_type = other DNA
aaaccccaaaaaaaaaaaaaaaaaaaaaaaaaaaaaaaaaaaaaaaaaaa

SEQ ID NO: 30 - DNA, 50 bp, synthetic construct
  misc_feature 1..50: note = Synthetic
  source 1..50: mol_type = other DNA
aaaaaaccccaaaaaaaaaaaaaaaaaaaaaaaaaaaaaaaaaaaaaaaa

SEQ ID NO: 31 - DNA, 50 bp, synthetic construct
  misc_feature 1..50: note = Synthetic
  source 1..50: mol_type = other DNA
aaatacgcatacatcctaagaactcagactacctcccaataaatccacac

SEQ ID NO: 32 - DNA, 50 bp, synthetic construct
  misc_feature 1..50: note = Synthetic
  source 1..50: mol_type = other DNA
aaatcagactacctcccaataaatccgcagcaatcctcacacctaataat

SEQ ID NO: 33 - DNA, 50 bp, synthetic construct
  misc_feature 1..50: note = Synthetic
  source 1..50: mol_type = other DNA
ccctacgcatacatcctaagaactcagactacctcccaataaatccacac

SEQ ID NO: 34 - DNA, 50 bp, synthetic construct
  misc_feature 1..50: note = Synthetic
  source 1..50: mol_type = other DNA
ccctcagactacctcccaataaatccgcagcaatcctcacacctaataat

SEQ ID NO: 35 - DNA, 50 bp, synthetic construct; identical to SEQ ID NO: 15
  misc_feature 1..50: note = Synthetic
  source 1..50: mol_type = other DNA

SEQ ID NO: 36 - DNA, 50 bp, synthetic construct; identical to SEQ ID NO: 16
  misc_feature 1..50: note = Synthetic
  source 1..50: mol_type = other DNA

SEQ ID NO: 37 - DNA, 50 bp, synthetic construct
  misc_feature 1..50: note = Synthetic
  source 1..50: mol_type = other DNA
accccccccccccccccccccccccccccccccccccccccccccccccc

SEQ ID NO: 38 - DNA, 50 bp, synthetic construct
  misc_feature 1..50: note = Synthetic
  source 1..50: mol_type = other DNA
cacccccccccccccccccccccccccccccccccccccccccccccccc

SEQ ID NO: 39 - DNA, 50 bp, synthetic construct; identical to SEQ ID NO: 21
  misc_feature 1..50: note = Synthetic
  source 1..50: mol_type = other DNA

SEQ ID NO: 40 - DNA, 50 bp, synthetic construct; identical to SEQ ID NO: 22
  misc_feature 1..50: note = Synthetic
  source 1..50: mol_type = other DNA

SEQ ID NO: 41 - DNA, 50 bp, synthetic construct; identical to SEQ ID NO: 24
  misc_feature 1..50: note = Synthetic
  source 1..50: mol_type = other DNA

SEQ ID NO: 42 - DNA, 50 bp, synthetic construct; identical to SEQ ID NO: 25
  misc_feature 1..50: note = Synthetic
  source 1..50: mol_type = other DNA

SEQ ID NO: 43 - DNA, 50 bp, synthetic construct
  misc_feature 1..50: note = Synthetic
  source 1..50: mol_type = other DNA
gaaaaaaaaaaaaaaaaaaaaaaaaaaaaaaaaaaaaaaaaaaaaaaaaa

SEQ ID NO: 44 - DNA, 50 bp, synthetic construct
  misc_feature 1..50: note = Synthetic
  source 1..50: mol_type = other DNA
agaaaaaaaaaaaaaaaaaaaaaaaaaaaaaaaaaaaaaaaaaaaaaaaa

SEQ ID NO: 45 - DNA, 50 bp, synthetic construct
  misc_feature 1..50: note = Synthetic
  source 1..50: mol_type = other DNA
aagaaaaaaaaaaaaaaaaaaaaaaaaaaaaaaaaaaaaaaaaaaaaaaa

SEQ ID NO: 46 - DNA, 84 bp, synthetic construct
  misc_feature 1..84: note = Synthetic
  source 1..84: mol_type = other DNA
tctggctctgttgctctctcgcaacagagccagaaaaaaaaaaaaaaaaaaaaaaaaaaaaaaaaaaaaaaaaaaaaaaaaaaa

SEQ ID NO: 47 - DNA, 84 bp, synthetic construct
  misc_feature 1..84: note = Synthetic
  source 1..84: mol_type = other DNA
cctggctctgttgctctctcgcaacagagccaggaaaaaaaaaaaaaaaaaaaaaaaaaaaaaaaaaaaaaaaaaaaaaaaaaa

SEQ ID NO: 48 - DNA, 84 bp, synthetic construct
  misc_feature 1..84: note = Synthetic
  source 1..84: mol_type = other DNA
actggctctgttgctctctcgcaacagagccagtaaaaaaaaaaaaaaaaaaaaaaaaaaaaaaaaaaaaaaaaaaaaaaaaaa

SEQ ID NO: 49 - DNA, 84 bp, synthetic construct
  misc_feature 1..84: note = Synthetic
  source 1..84: mol_type = other DNA
gccggctctggtgctctctcgcaccagagccggcaaaaaaaaaaaaaaaaaaaaaaaaaaaaaaaaaaaaaaaaaaaaaaaaaa

SEQ ID NO: 50 - DNA, 80 bp, synthetic construct
  misc_feature 1..80: note = Synthetic
  source 1..80: mol_type = other DNA
gctgtctgttgctctctcgcaacagacagcaaaaaaaaaaaaaaaaaaaaaaaaaaaaaaaaaaaaaaaaaaaaaaaaaa

SEQ ID NO: 51 - DNA, 76 bp, synthetic construct
  misc_feature 1..76: note = Synthetic
  source 1..76: mol_type = other DNA
gctctgttgctctctcgcaacagagcaaaaaaaaaaaaaaaaaaaaaaaaaaaaaaaaaaaaaaaaaaaaaaaaaa

SEQ ID NO: 52 - DNA, 72 bp, synthetic construct
  misc_feature 1..72: note = Synthetic
  source 1..72: mol_type = other DNA
gctgttgctctctcgcaacagcaaaaaaaaaaaaaaaaaaaaaaaaaaaaaaaaaaaaaaaaaaaaaaaaaa

SEQ ID NO: 53 - DNA, 100 bp, synthetic construct
  misc_feature 1..100: note = Synthetic
  source 1..100: mol_type = other DNA
aaaaaaaaaaaaaaaaaaaaaaaaaaaaaaaaaaaaaaaaaaaaaaaaaaaaaaaaaaaaaaaaaaaaaaaaaaaaaaaaaaaaaaaaaaaaaaaaaaaa

SEQ ID NO: 54 - DNA, 50 bp, synthetic construct; identical to SEQ ID NO: 27
  misc_feature 1..50: note = Synthetic
  source 1..50: mol_type = other DNA

SEQ ID NO: 55 - skipped